European Patent Specification EP 4 126 088 B1, published July 30, 2025. Title: COLLAGEN-BASED FORMULATIONS USABLE AS SOFT TISSUE FILLERS AND/OR IMPLANTS. Applicant: CollPlant Ltd. ORR, Nadav STERN, Miriam ZARKA, Revital. The sequence listing filed with the application follows.

SEQUENCE LISTING (7 sequences)

SEQ ID NO: 1 - DNA, 4662 bp, Artificial Sequence - collagen alpha chain 1
  "Synthetic sequence containing the coding regions of the vacuolar signal sequence of barley gene for Thiol protease aleurain precursor fused to the human Collagen alpha 1(I) chain and flanking regions"
gcgatgcatgtaatgtcatgagccacatgatccaatggccacaggaacgtaagaatgtagatagatttgattttgtccgttagatagcaaacaacattataaaaggtgtgtatcaatacgaactaattcactcattggattcatagaagtccattcctcctaagtatctaaaccatggctcacgctcgtgttctcctcctcgctctcgctgttttggcaacagctgctgtggctgtggcttctagttcttcttttgctgattcaaaccctattagacctgttactgatagagcagcttccactttggctcaattgcaagaggagggccaggttgagggccaagatgaggatatccctccaattacatgcgtgcaaaatggcttgcgttaccacgatagggatgtgtggaaacctgaaccttgtcgtatctgtgtgtgtgataacggcaaggtgctctgcgatgatgttatctgcgatgagacaaaaaattgccctggcgctgaagttcctgagggcgagtgttgccctgtgtgccctgatggttccgagtccccaactgatcaggaaactactggcgtggagggcccaaaaggagatactggtccacgtggtcctaggggtccagcaggtcctccaggtagagatggtattccaggccagcctggattgccaggaccaccaggcccacctggcccaccaggacctcctggtcttggtggaaatttcgctccacaactctcttatggctatgatgagaagtcaacaggtggtatttccgttccaggtcctatgggaccatccggaccaagaggtctcccaggtcctccaggtgctcctggacctcaaggctttcaaggacctccaggcgaaccaggagaaccaggcgcttctggaccaatgggcccaaggggaccacctggcccaccaggaaaaaatggcgatgatggcgaagctggaaagcctggtcgtcctggagagagaggtcctcctggcccacagggtgcaagaggcttgccaggaactgctggcttgcctggaatgaagggacataggggcttctccggcctcgatggcgctaagggtgatgctggccctgctggaccaaagggcgagccaggttcccctggagaaaacggtgctcctggacaaatgggtcctcgtggacttccaggagaaaggggtcgtccaggcgctccaggaccagcaggtgctaggggaaacgatggtgcaacaggcgctgctggccctcctggcccaactggtcctgctggccctccaggattcccaggcgcagttggagctaaaggagaagcaggaccacagggccctaggggttctgaaggacctcagggtgttagaggtgaaccaggtcctccaggcccagctggagcagctggtccagcaggaaatccaggtgctgatggtcaacctggagctaagggcgctaatggcgcaccaggtatcgcaggcgcaccaggttttcctggcgctagaggcccaagtggtcctcaaggaccaggtggaccaccaggtccaaaaggcaattctggcgaacctggcgctccaggttctaaaggagatactggtgctaaaggcgaaccaggacctgttggtgttcagggtcctcctggtcctgctggagaagaaggaaaaagaggtgctcgtggagaaccaggaccaactggacttcctggacctcctggtgaacgtggcggacctggctcaaggggtttccctggagctgatggagtggcaggtccaaaaggccctgctggagagagaggttcaccaggtccagctggtcctaagggctcccctggtgaagcaggtagaccaggcgaagcaggattgccaggcgcaaagggattgacaggctctcctggtagtcctggcccagatggaaaaacaggcccaccaggtccagcaggacaagatggacgtccaggcccaccaggtcctcctggagcaaggggacaagctggcgttatgggttttccaggacctaaaggtgctgctggagagccaggaaaggcaggtgaaagaggagttcctggtccaccaggagcagtgggtcctgctggcaaagatggtgaagctggagcacagggccctccaggccctgctggcccagctggcgaacgtggagaacaaggcccagctggtagtccaggatttcaaggattgcctggccctgctggccctccaggagaagcaggaaaacctggagaacaaggagttcctggtgatttgggagcacctggaccttcaggagcacgtggtgaaagaggcttccctggcgagaggggtgttcaaggtccaccaggtccagcaggacctagaggtgctaatggcgctcctggcaacgatggagcaaaaggtgatgctggtgctcctggcgcacctggaagtcagggtgctcctggattgcaaggaatgcctggagagaggggtgctgctggcttgccaggcccaaagggcgataggggtgatgctggaccaaaaggtgctgatggatccccaggaaaagatggagttcgtggtcttactggcccaatcggacctccaggccctgctggcgctccaggtgataagggcgaaagtggcccaagtggacctgctggacctactggtgctagaggtgcacctggtgataggggtgaacctggaccacctggtccagctggttttgctggtcctcctggagctgatggacaacctggcgcaaagggtgaaccaggtgatgctggcgcaaagggagatgctggtccacctggacctgctggtccagcaggcccccctgggccaatcggtaatgttggagcaccaggtgctaagggagctaggggttccgctggtccacctggagcaacaggatttccaggcgctgctggtagagttggcccaccaggcccatccggaaacgcaggccctcctggtcctccaggtcctgctggcaaggagggtggcaaaggaccaaggggcgaaactggccctgctggtagacctggcgaagttggccctcctggaccaccaggtccagcaggagaaaaaggttccccaggagctgatggcccagctggtgctccaggaactccaggccctcaaggtattgctggacagagaggcgttgtgggactccctggtcaaaggggagagagaggatttccaggcttgccaggacctagtggagaacctggaaaacaaggcccatcaggcgctagtggagagcgtggacctcctggccctatgggacctcctggattggctggcccacctggcgaatcaggtcgtgaaggcgcaccaggcgcagaaggatcacctggaagagatggatcccctggtgctaaaggcgatcgtggagaaactggtccagcaggcccaccaggcgcaccaggtgcacctggcgctccaggacctgtgggaccagctggaaaatccggagataggggcgagacaggcccagcaggaccagctggacctgttggccctgctggcgctcgtggaccagcaggacctcaaggaccaaggggagataagggagaaacaggcgaacaaggcgataggggcattaagggtcataggggttttagtggcctccagggtcctcctggcccacctggatcaccaggagaacagggaccatctggtgcttccggcccagctggtccaagaggacctccaggatcagctggtgcacctggaaaagatggtcttaacggtctcccaggaccaatcggccctccaggacctagaggaagaacaggagatgctggccctgttggccctccaggacctcctggtccaccaggtccacctggtcctccatcagctggattcgatttttcatttcttccacagccaccacaagagaaagctcacgatggcggcagatattaccgtgctgatgatgctaacgttgttagggatagagatttggaagtggatacaactttgaaatccctctcccagcaaattgaaaacattagatctccagaaggttcacgtaaaaacccagctagaacatgtcgtgatttgaaaatgtgtcactccgattggaaaagtggtgaatactggattgatccaaatcagggctgtaatctcgatgctatcaaagttttctgtaacatggaaacaggcgaaacatgcgtttatcctactcaaccttccgtggctcagaaaaattggtacatctcaaaaaatcctaaagataagaggcacgtttggttcggtgaaagtatgactgatggatttcaatttgagtacggcggtcaaggtagtgatccagctgatgtggctattcaactcacatttttgcgtcttatgtccacagaggcatcacaaaacatcacttaccactgcaaaaacagtgtggcttatatggatcaacaaacaggaaaccttaagaaggctcttcttttgaagggctcaaacgagattgagattagagcagagggcaactcaaggtttacttattcagttactgttgatggctgcacttcacatactggcgcttggggtaaaacagttatcgagtataagactacaaaaacatcaagactcccaatcattgatgttgctcctctcgatgttggcgctcctgatcaagagttcggttttgatgtgggcccagtttgtttcctctaatgagctcgcggccgcatc

SEQ ID NO: 2 - DNA, 4362 bp, Artificial Sequence - collagen alpha chain 2
  "Synthetic sequence containing the coding regions of the vacuolar signal sequence of barley gene for Thiol protease aleurain precursor fused to the human Collagen alpha 2(I) chain and flanking regions"
gcgatgcatgtaatgtcatgagccacatgatccaatggccacaggaacgtaagaatgtagatagatttgattttgtccgttagatagcaaacaacattataaaaggtgtgtatcaatacgaactaattcactcattggattcatagaagtccattcctcctaagtatctaaaccatggctcacgctcgtgttctcctcctcgctctcgctgttttggcaacagctgctgtggctgtggcttcaagttctagttttgctgattccaacccaattcgtccagttactgatagagcagcttccactttggctcaattgcttcaagaagaaactgtgaggaagggccctgctggcgataggggccctaggggcgaaaggggtccaccaggacctccaggcagggatggcgaagatggtccaactggccctcctggacctcctggccctccagggccacccggcttgggcggaaacttcgcagctcaatacgatggcaagggtgttggtcttggtcctggtcctatgggcttgatgggacctagaggcccacctggtgctgctggtgctcctggaccacagggttttcagggaccagctggcgagccaggagagccaggccaaacaggaccagctggtgcaaggggacctgctggacctcctggaaaagctggtgaagatggtcacccaggcaaaccaggacgtcctggcgaaagaggtgttgttggaccacaaggcgctaggggatttccaggtacacctggattgccaggttttaagggcattcgtggtcataacggcctcgatggattgaagggacagcctggcgcacctggcgttaagggtgaacctggagcaccaggtgaaaacggtactcctggccagactggtgcaagaggactcccaggtgaaaggggtagagttggtgctcctggacctgctggagctaggggtagtgatggtagtgttggtcctgtgggccctgctggtccaatcggttccgctggcccacctggattcccaggcgctccaggacctaaaggagaaatcggtgctgtgggtaacgcaggtcctactggtccagcaggtcctcgtggagaagtgggattgccaggactttctggtccagtgggccctccaggcaaccctggagctaacggcttgacaggagctaaaggcgcagcaggactccctggagtggctggcgcaccaggattgcctggtccaaggggtatcccaggccctgttggcgcagctggagctactggtgcacgtggacttgttggcgaaccaggccctgctggatcaaaaggcgagtctggaaataagggagaacctggttctgctggacctcaaggtcctcctggaccttctggagaagaaggaaaaaggggaccaaatggcgaggctggatcagcaggtccaccaggaccacctggacttcgtggatcccctggtagtagaggacttccaggcgctgatggtagagcaggcgttatgggaccaccaggaagtagaggagcatccggtccagcaggagttaggggtcctaacggagatgctggtagaccaggtgaaccaggtcttatgggcccaaggggcctcccaggtagtccaggaaatatcggccctgctggaaaagaaggccctgttggacttccaggtattgatggacgtcctggccctattggcccagcaggtgcaagaggagaacctggcaatattggatttccaggaccaaagggtccaacaggcgatcctggaaaaaatggagataagggtcatgctggattggcaggcgcaaggggcgctcctggtccagatggaaacaacggcgcacagggtccacctggccctcagggtgttcaaggcggaaaaggcgaacaaggcccagctggaccaccaggctttcaaggcttgccaggaccaagtggtccagcaggtgaagttggcaagccaggcgagcgtggacttcatggcgagtttggactccctggaccagcaggaccaaggggtgaaagaggccctcctggagagagtggcgctgctggaccaacaggcccaatcggtagtagaggtcctagtggacctccaggcccagatggaaataagggtgaaccaggagttgtgggcgctgttggaacagctggtccttcaggaccatcaggactcccaggcgagagaggcgctgctggcattcctggaggaaaaggtgaaaaaggcgaacctggcctccgtggcgaaatcggaaatcctggacgtgatggtgctcgtggtgcacacggcgctgtgggcgctccaggccctgctggtgctactggtgatagaggagaggctggcgcagctggcccagcaggtcctgctggcccaaggggtagtcctggtgaaagaggcgaagttggacctgctggccctaacggctttgctggccctgctggagcagcaggtcaacctggcgctaaaggtgaaaggggcggaaagggcccaaaaggtgaaaatggcgttgtgggaccaactggtccagtgggcgcagctggacctgctggtccaaatggaccaccaggaccagcaggtagtagaggagatggtggacctccaggaatgacaggttttccaggtgctgctggtagaacaggacctcctggtcctagtggtatttctggtccaccaggaccaccaggtcctgctggaaaagaaggattgaggggtccacgtggtgatcaaggaccagtgggcagaactggtgaagttggcgcagtgggaccacctggttttgctggagaaaagggcccttctggagaggcaggaacagctggtcctcctggtacacctggacctcaaggacttttgggtgcacctggtattctcggattgccaggaagtaggggcgaacgtggacttcctggcgtggcaggagcagttggagaacctggccctctcggaatcgcaggcccaccaggcgcaagaggaccaccaggagctgttggatcaccaggcgtgaatggtgcacctggcgaggctggtcgtgatggaaacccaggaaatgatggcccaccaggaagagatggtcaacctggacacaaaggcgagaggggctacccaggaaatattggcccagttggtgctgctggcgcaccaggcccacacggtccagttggaccagcaggaaaacacggtaatcgtggcgaaacaggcccttcaggcccagtgggacctgctggtgctgttggcccaagaggaccatctggacctcaaggcattagaggcgataagggagagcctggcgaaaaaggacctagaggcttgcctggttttaaaggacacaacggtctccaaggacttccaggtatcgctggtcatcatggagatcagggtgctcctggatcagtgggtccagcaggtcctagaggcccagcaggcccttccggtccagcaggaaaggatggacgtactggccaccctggaactgtgggccctgctggaattagaggtcctcaaggtcatcagggccctgctggccctccaggtccaccaggtcctccaggcccaccaggagtttcaggtggtggttacgattttggttacgatggtgatttttaccgtgctgatcaacctagaagtgctccttctctccgtcctaaagattatgaagttgatgctactttgaaatcacttaacaaccagattgagactcttctcacacctgagggatcaagaaagaatccagcacgtacatgccgtgatctcagacttagtcacccagagtggtcaagtggctattattggattgatcctaatcagggttgtacaatggaggctatcaaagtttactgtgattttccaactggagagacatgtattagggcacaacctgagaacattccagctaaaaattggtatcgttcctctaaagataagaaacatgtttggctcggagagactattaacgctggttctcagttcgagtataatgttgagggcgttacttctaaagagatggcaactcagctcgcttttatgagattgctcgctaactacgcatcccaaaacatcacttatcactgcaaaaattccattgcatatatggatgaggagacaggaaatttgaagaaagcagttattctccaaggtagtaacgatgttgagcttgtggctgagggaaatagtagattcacttacacagttttggtggatggatgctcaaagaaaactaatgagtggggcaagacaatcattgagtacaagacaaataagccttctaggctcccatttctcgatattgcacctcttgatatcggaggagctgatcacgagttttttgttgatatcggacctgtttgttttaagtaatgagctcgcggccgcatc

SEQ ID NO: 3 - protein, 1489 aa, Artificial Sequence - collagen alpha 1
  human collagen alpha-1 chain
MAHARVLLLALAVLATAAVAVASSSSFADSNPIRPVTDRAASTLAQLQEEGQVEGQDEDIPPITCVQNGLRYHDRDVWKPEPCRICVCDNGKVLCDDVICDETKNCPGAEVPEGECCPVCPDGSESPTDQETTGVEGPKGDTGPRGPRGPAGPPGRDGIPGQPGLPGPPGPPGPPGPPGLGGNFAPQLSYGYDEKSTGGISVPGPMGPSGPRGLPGPPGAPGPQGFQGPPGEPGEPGASGPMGPRGPPGPPGKNGDDGEAGKPGRPGERGPPGPQGARGLPGTAGLPGMKGHRGFSGLDGAKGDAGPAGPKGEPGSPGENGAPGQMGPRGLPGERGRPGAPGPAGARGNDGATGAAGPPGPTGPAGPPGFPGAVGAKGEAGPQGPRGSEGPQGVRGEPGPPGPAGAAGPAGNPGADGQPGAKGANGAPGIAGAPGFPGARGPSGPQGPGGPPGPKGNSGEPGAPGSKGDTGAKGEPGPVGVQGPPGPAGEEGKRGARGEPGPTGLPGPPGERGGPGSRGFPGADGVAGPKGPAGERGSPGPAGPKGSPGEAGRPGEAGLPGAKGLTGSPGSPGPDGKTGPPGPAGQDGRPGPPGPPGARGQAGVMGFPGPKGAAGEPGKAGERGVPGPPGAVGPAGKDGEAGAQGPPGPAGPAGERGEQGPAGSPGFQGLPGPAGPPGEAGKPGEQGVPGDLGAPGPSGARGERGFPGERGVQGPPGPAGPRGANGAPGNDGAKGDAGAPGAPGSQGAPGLQGMPGERGAAGLPGPKGDRGDAGPKGADGSPGKDGVRGLTGPIGPPGPAGAPGDKGESGPSGPAGPTGARGAPGDRGEPGPPGPAGFAGPPGADGQPGAKGEPGDAGAKGDAGPPGPAGPAGPPGPIGNVGAPGAKGARGSAGPPGATGFPGAAGRVGPPGPSGNAGPPGPPGPAGKEGGKGPRGETGPAGRPGEVGPPGPPGPAGEKGSPGADGPAGAPGTPGPQGIAGQRGVVGLPGQRGERGFPGLPGPSGEPGKQGPSGASGERGPPGPMGPPGLAGPPGESGREGAPGAEGSPGRDGSPGAKGDRGETGPAGPPGAPGAPGAPGPVGPAGKSGDRGETGPAGPAGPVGPAGARGPAGPQGPRGDKGETGEQGDRGIKGHRGFSGLQGPPGPPGSPGEQGPSGASGPAGPRGPPGSAGAPGKDGLNGLPGPIGPPGPRGRTGDAGPVGPPGPPGPPGPPGPPSAGFDFSFLPQPPQEKAHDGGRYYRADDANVVRDRDLEVDTTLKSLSQQIENIRSPEGSRKNPARTCRDLKMCHSDWKSGEYWIDPNQGCNLDAIKVFCNMETGETCVYPTQPSVAQKNWYISKNPKDKRHVWFGESMTDGFQFEYGGQGSDPADVAIQLTFLRLMSTEASQNITYHCKNSVAYMDQQTGNLKKALLLKGSNEIEIRAEGNSRFTYSVTVDGCTSHTGAWGKTVIEYKTTKTSRLPIIDVAPLDVGAPDQEFGFDVGPVCFL

SEQ ID NO: 4 - protein, 1389 aa, Artificial Sequence - collagen alpha 2
  human collagen alpha-2 chain
MAHARVLLLALAVLATAAVAVASSSSFADSNPIRPVTDRAASTLAQLLQEETVRKGPAGDRGPRGERGPPGPPGRDGEDGPTGPPGPPGPPGPPGLGGNFAAQYDGKGVGLGPGPMGLMGPRGPPGAAGAPGPQGFQGPAGEPGEPGQTGPAGARGPAGPPGKAGEDGHPGKPGRPGERGVVGPQGARGFPGTPGLPGFKGIRGHNGLDGLKGQPGAPGVKGEPGAPGENGTPGQTGARGLPGERGRVGAPGPAGARGSDGSVGPVGPAGPIGSAGPPGFPGAPGPKGEIGAVGNAGPTGPAGPRGEVGLPGLSGPVGPPGNPGANGLTGAKGAAGLPGVAGAPGLPGPRGIPGPVGAAGATGARGLVGEPGPAGSKGESGNKGEPGSAGPQGPPGPSGEEGKRGPNGEAGSAGPPGPPGLRGSPGSRGLPGADGRAGVMGPPGSRGASGPAGVRGPNGDAGRPGEPGLMGPRGLPGSPGNIGPAGKEGPVGLPGIDGRPGPIGPAGARGEPGNIGFPGPKGPTGDPGKNGDKGHAGLAGARGAPGPDGNNGAQGPPGPQGVQGGKGEQGPAGPPGFQGLPGPSGPAGEVGKPGERGLHGEFGLPGPAGPRGERGPPGESGAAGPTGPIGSRGPSGPPGPDGNKGEPGVVGAVGTAGPSGPSGLPGERGAAGIPGGKGEKGEPGLRGEIGNPGRDGARGAHGAVGAPGPAGATGDRGEAGAAGPAGPAGPRGSPGERGEVGPAGPNGFAGPAGAAGQPGAKGERGGKGPKGENGVVGPTGPVGAAGPAGPNGPPGPAGSRGDGGPPGMTGFPGAAGRTGPPGPSGISGPPGPPGPAGKEGLRGPRGDQGPVGRTGEVGAVGPPGFAGEKGPSGEAGTAGPPGTPGPQGLLGAPGILGLPGSRGERGLPGVAGAVGEPGPLGIAGPPGARGPPGAVGSPGVNGAPGEAGRDGNPGNDGPPGRDGQPGHKGERGYPGNIGPVGAAGAPGPHGPVGPAGKHGNRGETGPSGPVGPAGAVGPRGPSGPQGIRGDKGEPGEKGPRGLPGFKGHNGLQGLPGIAGHHGDQGAPGSVGPAGPRGPAGPSGPAGKDGRTGHPGTVGPAGIRGPQGHQGPAGPPGPPGPPGPPGVSGGGYDFGYDGDFYRADQPRSAPSLRPKDYEVDATLKSLNNQIETLLTPEGSRKNPARTCRDLRLSHPEWSSGYYWIDPNQGCTMEAIKVYCDFPTGETCIRAQPENIPAKNWYRSSKDKKHVWLGETINAGSQFEYNVEGVTSKEMATQLAFMRLLANYASQNITYHCKNSIAYMDEETGNLKKAVILQGSNDVELVAEGNSRFTYTVLVDGCSKKTNEWGKTIIEYKTNKPSRLPFLDIAPLDIGGADHEFFVDIGPVCFK

SEQ ID NO: 5 - DNA, 1633 bp, Artificial Sequence - P4H
  "Synthetic sequence containing the coding regions of the vacuolar signal sequence of barley gene for Thiol protease aleurain precursor fused to the human Prolyl 4-hydroxylase beta subunit and flanking regions"
ctcgagtaaaccatggctcatgctagggttttgcttttggctcttgctgttcttgctactgctgctgttgctgtggcttcttcttcatctttcgctgattctaacccaattaggccagtgactgatagagctgcttctactcttgctcaattggtcgacatggatgctccagaagaggaggatcacgttcttgtgcttaggaagtctaacttcgctgaagctcttgctgctcacaagtaccttcttgtggagttttatgctccttggtgcggacattgcaaagctcttgctccagagtatgctaaggctgctggaaagttgaaggctgagggatctgaaattaggcttgctaaagtggatgctactgaggagtctgatcttgctcaacagtacggagttaggggatacccaactattaagttcttcaggaacggagatactgcttctccaaaggagtatactgctggaagggaggctgatgatattgtgaactggcttaagaagagaactggaccagctgctactactcttccagatggagctgctgctgaatctcttgtggagtcatctgaggtggcagtgattggattcttcaaggatgtggagtctgattctgctaagcagttccttcaagctgctgaggctattgatgatattccattcggaattacttctaactctgatgtgttctctaagtaccagcttgataaggatggagtggtgcttttcaagaaattcgatgagggaaggaacaatttcgagggagaggtgacaaaggagaaccttcttgatttcattaagcacaaccagcttccacttgtgattgagttcactgagcagactgctccaaagattttcggaggagagattaagactcacattcttcttttccttccaaagtctgtgtctgattacgatggaaagttgtctaacttcaagactgctgctgagtctttcaagggaaagattcttttcattttcattgattctgatcacactgataaccagaggattcttgagttcttcggacttaagaaggaagagtgcccagctgttaggcttattactcttgaggaggagatgactaagtacaagccagagtctgaagaacttactgctgagaggattactgagttctgccacagattccttgagggaaagattaagccacaccttatgtctcaagagcttccagaggattgggataagcagccagttaaggtgttggtgggtaaaaacttcgaggatgtggctttcgatgagaagaagaacgtgttcgtggagttctacgcaccttggtgtggtcactgtaagcagcttgctccaatttgggataagttgggagagacttacaaggatcacgagaacattgtgattgctaagatggattctactgctaacgaggtggaggctgttaaggttcactctttcccaactttgaagttcttcccagcttctgctgataggactgtgattgattacaacggagaaaggactcttgatggattcaagaagttccttgagtctggaggacaagatggagctggagatgatgatgatcttgaggatttggaagaagctgaggagccagatatggaggaggatgatgatcagaaggctgtgtgatgagctc

SEQ ID NO: 6 - DNA, 1723 bp, Artificial Sequence - P4H
  "Synthetic sequence containing the coding regions of the vacuolar signal sequence of barley gene for Thiol protease aleurain precursor fused to the human Prolyl 4-hydroxylase alpha-1 subunit and flanking regions"
ctcgagtaaaccatggctcatgctagggttttgcttttggctcttgctgttcttgctactgctgctgttgctgtggcttcttcttcatctttcgctgattctaacccaattaggccagtgactgatagagctgcttctactcttgctcaattggtcgacatgcacccaggattcttcacttctattggacagatgactgatcttattcacactgagaaggatcttgtgacttctcttaaggattacattaaggctgaggaggataagttggagcagattaagaagtgggctgagaagttggataggcttacttctactgctacaaaagatccagagggattcgttggtcatccagtgaacgctttcaagttgatgaagaggcttaacactgagtggagtgagcttgagaaccttgtgcttaaggatatgtctgatggattcatttctaaccttactattcagaggcagtacttcccaaatgatgaggatcaagtgggagctgctaaggctcttcttaggcttcaggatacttacaaccttgatactgatacaatttctaagggaaaccttccaggagttaagcacaagtctttccttactgctgaggattgcttcgagcttggaaaggttgcatacactgaggctgattactaccacactgagctttggatggaacaagctcttaggcaacttgatgagggagagatttctactattgataaggtgtcagtgcttgattacctttcttacgctgtgtaccagcagggtgatcttgataaggctcttttgcttactaagaagttgcttgagcttgatccagaacatcagagggctaacggaaaccttaagtacttcgagtacattatggctaaggaaaaggatgtgaacaagtctgcttctgatgatcagtctgatcaaaagactactccaaagaagaagggagtggctgttgattatcttcctgagaggcagaagtatgagatgttgtgtaggggagagggtattaagatgactccaaggaggcagaagaagttgttctgcaggtatcacgatggaaacaggaacccaaagttcattcttgctccagctaagcaagaagatgagtgggataagccaaggattattaggttccacgatattatttctgatgctgagattgagattgtgaaggatcttgctaagccaagacttaggagggctactatttctaaccctattactggtgatcttgagactgtgcactacaggatttctaagtctgcttggctttctggatacgagaacccagtggtgtctaggattaacatgaggattcaggatcttactggacttgatgtgtctactgctgaggagcttcaagttgctaactacggagttggaggacaatatgagccacacttcgatttcgctaggaaggatgagccagatgcttttaaggagcttggaactggaaacaggattgctacttggcttttctacatgtctgatgtttctgctggaggagctactgttttcccagaagtgggagcttctgtttggccaaagaagggaactgctgtgttctggtacaaccttttcgcttctggagagggagattactctactaggcatgctgcttgcccagttcttgttggaaacaagtgggtgtcaaacaagtggcttcatgagaggggacaagagtttagaaggccatgcactctttctgagcttgagtgatgagctc

SEQ ID NO: 7 - DNA, 2888 bp, Artificial Sequence - LH3
  "Synthetic sequence containing the coding regions of the vacuolar signal sequence of barley gene for Thiol protease aleurain precursor fused to the human Lysyl hydroxylase 3 and flanking regions"
gcgaattcgctagctatcactgaaaagacagcaagacaatggtgtctcgatgcaccagaaccacatctttgcagcagatgtgaagcagccagagtggtccacaagacgcactcagaaaaggcatcttctaccgacacagaaaaagacaaccacagctcatcatccaacatgtagactgtcgttatgcgtcggctgaagataagactgaccccaggccagcactaaagaagaaataatgcaagtggtcctagctccactttagctttaataattatgtttcattattattctctgcttttgctctctatataaagagcttgtattttcatttgaaggcagaggcgaacacacacacagaacctccctgcttacaaaccagatcttaaaccatggctcacgctagggttttgcttcttgctcttgctgttcttgctactgctgctgttgctgtggcttcttcaagttctttcgctgattctaacccaattaggccagtgactgatagagctgcttctactcttgctcaattgagatctatgtctgatagaccaaggggaagggatccagttaatccagagaagttgcttgtgattactgtggctactgctgagactgaaggataccttagattccttaggagtgctgagttcttcaactacactgtgaggactcttggacttggagaagaatggaggggaggagatgttgctagaactgttggaggaggacagaaagtgagatggcttaagaaagagatggagaagtacgctgatagggaggatatgattattatgttcgtggattcttacgatgtgattcttgctggatctccaactgagcttttgaagaaattcgttcagtctggatctaggcttcttttctctgctgagtctttttgttggccagaatggggacttgctgagcaatatccagaagtgggaactggaaagagattccttaactctggaggattcattggattcgctactactattcaccagattgtgaggcagtggaagtacaaggatgacgatgatgatcagcttttctacactaggctttaccttgatccaggacttagggagaagttgtctcttaaccttgatcacaagtctaggattttccagaaccttaacggtgctcttgatgaggttgtgcttaagttcgataggaacagagtgaggattaggaacgtggcttacgatactcttcctattgtggtgcatggaaacggaccaacaaaactccagcttaactaccttggaaactacgttccaaacggatggactccagaaggaggatgtggattctgcaatcaggataggagaactcttccaggaggacaaccaccaccaagagttttccttgctgtgttcgttgaacagccaactccattccttccaagattccttcagaggcttcttcttttggattacccaccagatagggtgacacttttccttcacaacaacgaggttttccacgagccacacattgctgattcttggccacagcttcaggatcatttctctgctgtgaagttggttggtccagaagaagctctttctccaggagaagctagggatatggctatggatttgtgcaggcaggatccagagtgcgagttctacttctctcttgatgctgatgctgtgcttactaaccttcagactcttaggattcttattgaggagaacaggaaagtgattgctccaatgctttctaggcacggaaagttgtggtctaatttctggggtgctctttctcctgatgagtactacgctagatcagaggactacgtggagcttgttcagagaaagagagtgggagtttggaacgttccttatatttctcaggcttacgtgattaggggagatactcttaggatggagcttccacagagggatgttttctctggatctgatactgatccagatatggctttctgcaagtctttcagggataagggaattttccttcacctttctaaccagcatgagttcggaagattgcttgctacttcaagatacgatactgagcaccttcatcctgatctttggcagattttcgataacccagtggattggaaggagcagtacattcacgagaactactctagggctcttgaaggagaaggaattgtggagcaaccatgcccagatgtttactggttcccacttctttctgagcaaatgtgcgatgagcttgttgctgagatggagcattacggacaatggagtggaggtagacatgaggattctaggcttgctggaggatacgagaacgttccaactgtggatattcacatgaagcaagtgggatacgaggatcaatggcttcagcttcttaggacttatgtgggaccaatgactgagtctcttttcccaggataccacactaaggctagggctgttatgaacttcgttgtgaggtatcgtccagatgagcaaccatctcttaggccacaccacgattcttctactttcactcttaacgtggctcttaaccacaagggacttgattatgagggaggaggatgccgtttccttagatacgattgcgtgatttcttcaccaagaaagggatgggctcttcttcatccaggaaggcttactcattaccacgagggacttccaactacttggggaactagatatattatggtgtctttcgtggatccatgactgctttaatgagatatgcgagacgcctatgatcgcatgatatttgctttcaattctgttgtgcacgttgtaaaaaacctgagcatgtgtagctcagatccttaccgccggtttcggttcattctaatgaatatatcacccgttactatcgtatttttatgaataatattctccgttcaatttactgattgtccagaattcgcg